European Patent Specification EP 3 372 690 B1, published March 12, 2025. Title: Method of detecting chromosome abnormality in embryo by using blastocyst culture. Applicant: XUKANG MEDICAL SCIENCE & TECHNOLOGY (SUZHOU) CO., LTD. The sequence listing filed with the application follows.

SEQUENCE LISTING (6 sequences)

SEQ ID NO: 1 - DNA, 35 bp, artificial sequence
  primer
  misc_feature (28)..(35): n is a, c, g, or t
gtgagtgatggttgaggtagtgtggagnnnnnnnn

SEQ ID NO: 2 - DNA, 35 bp, artificial sequence
  primer
  misc_feature (28)..(32): n is a, c, g, or t
gtgagtgatggttgaggtagtgtggagnnnnnggg

SEQ ID NO: 3 - DNA, 35 bp, artificial sequence
  primer
  misc_feature (28)..(32): n is a, c, g, or t
gtgagtgatggttgaggtagtgtggagnnnnnttt

SEQ ID NO: 4 - DNA, 35 bp, artificial sequence
  primer
  misc_feature (28)..(30): n is a, c, g, or t
  misc_feature (32)..(32): n is a, c, g, or t
  misc_feature (34)..(34): n is a, c, g, or t
gtgagtgatggttgaggtagtgtggagnnntntng

SEQ ID NO: 5 - DNA, 36 bp, artificial sequence
  primer
  misc_feature (28)..(30): n is a, c, g, or t
  misc_feature (35)..(36): n is a, c, g, or t
gtgagtgatggttgaggtagtgtggagnnngtggnn

SEQ ID NO: 6 - DNA, 27 bp, artificial sequence
  primer
gtgagtgatggttgaggtagtgtggag